European Patent Specification EP 3 370 527 B1, published August 2, 2023. Title: Cotton Transgenic Event MON 88702 And Methods For Detection And Uses Thereof. Applicant: Monsanto Technology LLC. The sequence listing filed with the application follows.

SEQUENCE LISTING (27 sequences)

SEQ ID NO: 1 - DNA, 20 bp, Artificial
  A twenty nucleotide sequence representing the 5' junction regions of cotton genomic DNA and the integrated transgenic expression cassette.
aaaaaaatatagtcagcatc

SEQ ID NO: 2 - DNA, 20 bp, Artificial
  A twenty nucleotide sequence representing the 3' junction regions of cotton genomic DNA and the integrated trasngenic expression cassette.
ctttcttttttcaatataaa

SEQ ID NO: 3 - DNA, 60 bp, Artificial
  A sixty nucleotide sequence representing the 5' junction regions of cotton genomic DNA and the integrated transgenic expression cassette.
tatgaaagataaaataatagaaaaaaatatagtcagcatcatcacaccaaaagttaggcc

SEQ ID NO: 4 - DNA, 60 bp, Artificial
  A sixty nucleotide sequence representing the 3' junction regions of cotton genomic DNA and the integrated trasngenic expression cassette.
aaaaaaaattggtaattactctttcttttttcaatataaacatgggaaatttgaaacttc

SEQ ID NO: 5 - DNA, 100 bp, Artificial
  A one hundred nucleotide sequence representing the 5' junction regions of cotton genomic DNA and the integrated trasngenic expression cassette.
gaaatttcctcttttttcaatatgaaagataaaataatagaaaaaaatatagtcagcatcatcacaccaaaagttaggcccgaatagtttgaaattagaa

SEQ ID NO: 6 - DNA, 100 bp, Artificial
  A one hundred nucleotide sequence representing the 3' junction regions of cotton genomic DNA and the integrated trasngenic expression cassette.
acatctacatttttgaattgaaaaaaaattggtaattactctttcttttttcaatataaacatgggaaatttgaaacttcctttttattattctaagaag

SEQ ID NO: 7 - DNA, 1651 bp, Gossypium hirsutum
  misc_feature (1)..(1651): Nucleotide sequence representing the 5' flanking cotton genomic sequence up to the inserted T-DNA.
gttatatatataatttaaaactttttcctttggttggaataacaactaacattaaatttgaacctcttttattttcctctatagtttttcttttatggaaaagtgattgtacccttcttcaattgtaaaaaggtgaagggggaatcaatggtcatcttttgcttgattggtgcttctcccaaagtcatctaatcaaataaagatagagaaaaaaaaggggggagggacttgaaaaaagtatacttgctttgagtgcaagaagctaccaaaactttttagatggaccaaaaataaaaaaggtggtagccctaaaatctcccccccccccaagctgtgagtgacttgttatttttatgtttgcttaaagtttgacctttcatgacatgattatcacatacttgattgtatacatgtgtgtgtaaaaaagttaaatgtggggtttggcttgcactagtgaaaagaattatgggaccctttgtctcatgatataccatcaattatcccttggaagaggctcttttttaaattattgttattatttacatcaactatatgatcatggatggatcaattgtgattttgaactttgggggtgccttttttgatgttctaataactcaaataaaaacgagactctagcaattagatgatgagaagacaattaagggtgtttttttctttctgaagatccctttaaatggggtcattggttgatatctagcaatccttgaagcaaatatatatttatatattatatggagagagaaagcattttaaatgatggttcttatatcattgaggtatatagtgggagaatcatatttttccttgtgaaggaaccaacaacaaagcaagcaaacaccttttgataattatggtaagataaaataataataaggcataatgactaactaagctcttaacatttatatattctgtcgatttaatccttattcttttttgagctaaatttgactatcaacctttcaaaaataattgaatgttgccttttttttaatggaaatacaaactaaaacgttaaatttttaaacataacaacccaaatggcaatccatttgtatttcatactaattttttaaaattttaagaactttttatatatatattttttagattttgaattcgcttttattttttaatcatttgttaacataacgtatacaacaaaatagtgctatgtcagcatgaagtatatatggactgccatgtgggttgtcatgtcaacatagataaaaaattaattttttagtcagtatttccatttaaaagaaaaacaatttgactctttttaaaagactaatgatttaatttaactaaaaaaaataagggtcaaattgatcaaatatataaatattgagggctgaatttatcatcatacctaatactaatcttaagagagagagagagtggagatagatagaatgatgaaaagagatctaacaaggtttcaagtgtggggaaaaaaagtttaggctaatgagaccaccttttcttttttaattaattaaaaggaattagtatggtatcatatgcttaaggagtgggtatgcaaaagacaaaaacccaaggagcttccaccagaaatttcctcttttttcaatatgaaagataaaataatagaaaaaaatat

SEQ ID NO: 8 - DNA, 2010 bp, Gossypium hirsutum
  misc_feature (1)..(2010): Nucleotide sequence representing the 3' flanking cotton genomic sequence after the inserted T-DNA.
  misc_feature (1)..(4): The first four nucleotides of this sequence are derived from an unknown origin and are not present in the non-transgenic DP393 variety and were likely introduced during the integration of the MON 88702 T-DNA.
tcaatataaacatgggaaatttgaaacttcctttttattattctaagaagtattaattccataatgaatgcatgaaggagttgttcaacaaattaatgaccaaaggtgaaattaaaagatttgtactcagaaattaatttttaatttaagtcgtgagacacgcttttgaaatgcattgaagttttttttttttaattaaatacaaatttccagataatgttagggacaaggcaaactagatggaaagacagtcattgaactaataagtaacagtaagaatatgtgtctttctttttattataacatacaaacacttagacattattaaaacagcccaagtttgtcgtttacaaagattgcaatctccatatcatgacaatacaatatactccatattgattgcattcataaaatatcattttacctcccttaccttaaatcccattcattcattagcatgagatttcaagtaaaattatgaactgaaaattagccaaatttattcaaaatttgaagaaaaaaaaccattttttctaataatttagtggcttaaattaaatctttcgaataattgaatgaccaaaatgtaattttattaataatttaatgacattggatgtaatatactcaatctaatatatcgagttaaaaaaaaaattctttggtacaaccagtgagttgtgtgaaatgcttcttaattaactatatgttcaattatatacattcaaaaacatacaaaatagccctgaaatatccaactttaatgggaccaatattatttttcatctatcgtaacatactacaacagttctatcaaaacatacaaaaattattgtttttttcttttttttttactcaggacccgcttagttcgactcatgaactagtttattttggatgtatatttttttatataatttcagtaaaatatatttcaaacattattgaagcaaagcaagaatgtaagtggtagagcagacagtatgttcactgatactgatgtcatatatatatatgttgggatgcaaggtttatagtgataaacaagaggttgaagatgttgtgtaagcatggtgccaagggaaaacatgaagaattggaccaccttctttacatgaatttggctgcatccttattctaacccattaatatttaaattataaaatattgtcattaagataacatgtcatttccttctctcattttctctgccaaatttgttctttttctccttctttttttttttcctttccatgtcttttaaagttctgattttgagagctgtctcctctatcttttatcttatttacataaaataaataaatttcatcataaatttaagtcccccaaaaaataaaaccataaaataaaataaaatctcagaaaaacctcccgttcgaaagcctctttcttttcttccacgggagcttaaagcttcgtcttgcaaaagtgggatagcacgaacttttgtgtgctttgtattgttattaattcttatatatttgccgtcaatccttatattttgaaaaaaaatttatgatttaatctctgtatttaaaaggttaaattttaagtttttcttttttttttaatttaaaaatctcagtctaaccattaacattattaatatttttctatcaaaatttatgaatttagcattttaattagattgtcctcatatgtcatgatatattaagttgacaaattttgattaaaattactagcaacgataatgattggattaggattgttaaattaaaaaataagaattgcatttttaaaaatattttttaaactgaaccggtgatcaaattggtcagatcatcggttcacaggcctaatcgtctaatcgattcgattaaaaattaataaaaattcaaaaaaaaattaaaatctcaattcaaccagttctcaatctaatcagttcaaagccactttccggactaattcccccaatcgattcttggtccggtccaattcaaataatactaattttttacttttaaagca

SEQ ID NO: 9 - DNA, 3143 bp, Artificial
  Nucleotide sequence corresponding to the inserted T-DNA in cotton event MON 88702.
agtcagcatcatcacaccaaaagttaggcccgaatagtttgaaattagaaagctcgcaattgaggtctgtcgaccctgcactaactataacggtcctaaggtagcgatacactggcgcgccaattctcagtccaaagcctcaacaaggtcagggtacagagtctccaaaccattagccaaaagctacaggagatcaatgaagaatcttcaatcaaagtaaactactgttccagcacatgcatcatggtcagtaagtttcagaaaaagacatccaccgaagacttaaagttagtgggcatctttgaaagtaatcttgtcaacatcgagcagctggcttgtggggaccagacaaaaaaggaatggtgcagaattgttaggcgcacctaccaaaagcatctttgcctttattgcaaagataaagcagattcctctagtacaagtggggaacaaaataacgtggaaaagagctgtcctgacagcccactcactaatgcgtatgacgaacgcagtgacgaccacaaaagaattagcttgcctgcaggattagcttagatcgggcttaattaaggcgcgccggccaagtcggccgcggccgcaagcttacttgcgacagaaacagctttgatatattattactcacccgttatcgatatggaatatatactttaagaactcactaaatcatatccttcatgtcggtttaaagattagtcacgtatctgcacattctgtaagtatagtaatctcataaaaaacctggtctctgttctctgtgaatccataggttattgcactggcgtactactgtatatcatatttccctggtggatcatcgggaatgaagttcctcagttctactcttacctcctctgtcttccgaatgtttgggagatgagctttcgctttgacctatgcaaagaaaataacttgattctctcgtgtataaagaaagatgaaagatcttcaacagtggttaaatgacaaatctggtaaaatatgttggtccaatggctcaaagacagttttgttataaatttcctatattgatactttctgctaaattggttcaaaacttcaaatcactagccactggatgaggtatggaacttgaagagttgcttggtggatacattctctaatctagggtaagtcgttagcttcaatgtcttactgtgaattattacatcagaattaagaaagttattacacgtatgttttcactgagtttactacactggcaatgtggcatacatctcttactgcaaattgcagacaagtggtcaatcaaatcttttttagttgggcccaaaatgtctgttattggatacgttgggccttaaaatggcccccatcagtcaaaaacatcactgcttggagaaggatctagaaaaacttgcaagttagttcaaacaaaataaaggaaaaagaacgatctagaagaaagaaaaaaaaaggaaaagaaacccttatggaggttcccacaccactctatatataataacatccttctcctaaatcccgcatcagtacttctctctgctctcaagataattttgttctctcaatttcattcttaaaccctagttcttcgattttttccgatctacgacacctgcaggcctcagcgctgtgcctgttgcgatcgcccatggctatcctagaccttaagtccctcgtgctgaacgccattaactactggggccctaagaacaacaacggcatccagggcggtgacttcggctaccccatctctgagaagcagatcgacactagcatcattacctccacccaccctcgcttgatcccccacgatcttactatcccgcagaaccttgagaccatcttcaccacaacgcaggtgctcaccaataacactgacctccagcaatcccagaccgtgagctttgcgaagaagaccactaccacgaccgcaactagcacgaccaacggttggacagaaggaggcaagatcagcgacacgctggaggagaaagtttcggttagcattccgttcatcggtgagggtggcgggaagaactcgactaccatagaggccaacttcgcacacaactctagcaccactacctcccaggaagcaagcactgacattgagtggaacattagccaaccggtccttgtgcctccccgcaaacaggttgttgccactctcgttatcatgggtggcaacttcactattcctatggatcttatgactaccattgactctactgagcactactctggctaccccattctcacttggatctcttctcctgacaatagctacagcggtcgattcatgtcatggtacttcgctaactggccgaatctcccttctggctttggtcctcttaactctgataacactgtgacctacactggctctgtcgtcagtcaggtctctgccggtgtgtacgcaactgttcgcttcgatcagtatgacatccataatctctggactattgagaagacctggtacgctcgtcatgcgacgcttcacaacggcaagaagatcagcatcaataacgtgacagaaatggcccctaccagcccgatcaagactaactgagcgatcgccagcagaacacgcgctgagggcccaaatcaccagtctctctctacaaatctatctctctctatttttctccagaataatgtgtgagtagttcccagataagggaattagggttcttatagggtttcgctcatgtgttgagcatataagaaacccttagtatgtatttgtatttgtaaaatacttctatcaataaaatttctaattcctaaaaccaaaatccagtcaaatcctaccacctcatttaaatagagtgaggttgatttgcggccgcacgtcctgcttggcctactaggccaacgcaggcgctggccgtgacggccacgagcgaactaggccttgggccgcatcgatcgtgaagtttctcatctaagcccccatttggacgtgaatgtagacacgtcgaaataaagatttccgaattagaataatttgtttattgctttcgcctataaatacgacggatcgtaatttgtcgttttatcaaaatgtactttcattttataataacgctgcggacatctacatttttgaattgaaaaaaaattggtaattactctttcttttt

SEQ ID NO: 10 - DNA, 6804 bp, Artificial
  Nucleotide sequence corresponding to the contig nucleotide sequence of the 5' genomic flanking DNA nucleotide sequence, the inserted T-DNA nucleotide sequence in event MON 88702, and the 3' genomic flanking DNA nucleotide sequence.
  misc_feature (1)..(1651): The 5' genomic flanking sequence represented by SEQ ID NO: 7.
  misc_feature (1652)..(4794): The inserted T-DNA nucleotide sequence in event MON 88702 represented as SEQ ID NO: 9.
  misc_feature (4795)..(6804): The 3' genomic flanking DNA nucleotide sequence represented as SEQ ID NO: 8.
gttatatatataatttaaaactttttcctttggttggaataacaactaacattaaatttgaacctcttttattttcctctatagtttttcttttatggaaaagtgattgtacccttcttcaattgtaaaaaggtgaagggggaatcaatggtcatcttttgcttgattggtgcttctcccaaagtcatctaatcaaataaagatagagaaaaaaaaggggggagggacttgaaaaaagtatacttgctttgagtgcaagaagctaccaaaactttttagatggaccaaaaataaaaaaggtggtagccctaaaatctcccccccccccaagctgtgagtgacttgttatttttatgtttgcttaaagtttgacctttcatgacatgattatcacatacttgattgtatacatgtgtgtgtaaaaaagttaaatgtggggtttggcttgcactagtgaaaagaattatgggaccctttgtctcatgatataccatcaattatcccttggaagaggctcttttttaaattattgttattatttacatcaactatatgatcatggatggatcaattgtgattttgaactttgggggtgccttttttgatgttctaataactcaaataaaaacgagactctagcaattagatgatgagaagacaattaagggtgtttttttctttctgaagatccctttaaatggggtcattggttgatatctagcaatccttgaagcaaatatatatttatatattatatggagagagaaagcattttaaatgatggttcttatatcattgaggtatatagtgggagaatcatatttttccttgtgaaggaaccaacaacaaagcaagcaaacaccttttgataattatggtaagataaaataataataaggcataatgactaactaagctcttaacatttatatattctgtcgatttaatccttattcttttttgagctaaatttgactatcaacctttcaaaaataattgaatgttgccttttttttaatggaaatacaaactaaaacgttaaatttttaaacataacaacccaaatggcaatccatttgtatttcatactaattttttaaaattttaagaactttttatatatatattttttagattttgaattcgcttttattttttaatcatttgttaacataacgtatacaacaaaatagtgctatgtcagcatgaagtatatatggactgccatgtgggttgtcatgtcaacatagataaaaaattaattttttagtcagtatttccatttaaaagaaaaacaatttgactctttttaaaagactaatgatttaatttaactaaaaaaaataagggtcaaattgatcaaatatataaatattgagggctgaatttatcatcatacctaatactaatcttaagagagagagagagtggagatagatagaatgatgaaaagagatctaacaaggtttcaagtgtggggaaaaaaagtttaggctaatgagaccaccttttcttttttaattaattaaaaggaattagtatggtatcatatgcttaaggagtgggtatgcaaaagacaaaaacccaaggagcttccaccagaaatttcctcttttttcaatatgaaagataaaataatagaaaaaaatatagtcagcatcatcacaccaaaagttaggcccgaatagtttgaaattagaaagctcgcaattgaggtctgtcgaccctgcactaactataacggtcctaaggtagcgatacactggcgcgccaattctcagtccaaagcctcaacaaggtcagggtacagagtctccaaaccattagccaaaagctacaggagatcaatgaagaatcttcaatcaaagtaaactactgttccagcacatgcatcatggtcagtaagtttcagaaaaagacatccaccgaagacttaaagttagtgggcatctttgaaagtaatcttgtcaacatcgagcagctggcttgtggggaccagacaaaaaaggaatggtgcagaattgttaggcgcacctaccaaaagcatctttgcctttattgcaaagataaagcagattcctctagtacaagtggggaacaaaataacgtggaaaagagctgtcctgacagcccactcactaatgcgtatgacgaacgcagtgacgaccacaaaagaattagcttgcctgcaggattagcttagatcgggcttaattaaggcgcgccggccaagtcggccgcggccgcaagcttacttgcgacagaaacagctttgatatattattactcacccgttatcgatatggaatatatactttaagaactcactaaatcatatccttcatgtcggtttaaagattagtcacgtatctgcacattctgtaagtatagtaatctcataaaaaacctggtctctgttctctgtgaatccataggttattgcactggcgtactactgtatatcatatttccctggtggatcatcgggaatgaagttcctcagttctactcttacctcctctgtcttccgaatgtttgggagatgagctttcgctttgacctatgcaaagaaaataacttgattctctcgtgtataaagaaagatgaaagatcttcaacagtggttaaatgacaaatctggtaaaatatgttggtccaatggctcaaagacagttttgttataaatttcctatattgatactttctgctaaattggttcaaaacttcaaatcactagccactggatgaggtatggaacttgaagagttgcttggtggatacattctctaatctagggtaagtcgttagcttcaatgtcttactgtgaattattacatcagaattaagaaagttattacacgtatgttttcactgagtttactacactggcaatgtggcatacatctcttactgcaaattgcagacaagtggtcaatcaaatcttttttagttgggcccaaaatgtctgttattggatacgttgggccttaaaatggcccccatcagtcaaaaacatcactgcttggagaaggatctagaaaaacttgcaagttagttcaaacaaaataaaggaaaaagaacgatctagaagaaagaaaaaaaaaggaaaagaaacccttatggaggttcccacaccactctatatataataacatccttctcctaaatcccgcatcagtacttctctctgctctcaagataattttgttctctcaatttcattcttaaaccctagttcttcgattttttccgatctacgacacctgcaggcctcagcgctgtgcctgttgcgatcgcccatggctatcctagaccttaagtccctcgtgctgaacgccattaactactggggccctaagaacaacaacggcatccagggcggtgacttcggctaccccatctctgagaagcagatcgacactagcatcattacctccacccaccctcgcttgatcccccacgatcttactatcccgcagaaccttgagaccatcttcaccacaacgcaggtgctcaccaataacactgacctccagcaatcccagaccgtgagctttgcgaagaagaccactaccacgaccgcaactagcacgaccaacggttggacagaaggaggcaagatcagcgacacgctggaggagaaagtttcggttagcattccgttcatcggtgagggtggcgggaagaactcgactaccatagaggccaacttcgcacacaactctagcaccactacctcccaggaagcaagcactgacattgagtggaacattagccaaccggtccttgtgcctccccgcaaacaggttgttgccactctcgttatcatgggtggcaacttcactattcctatggatcttatgactaccattgactctactgagcactactctggctaccccattctcacttggatctcttctcctgacaatagctacagcggtcgattcatgtcatggtacttcgctaactggccgaatctcccttctggctttggtcctcttaactctgataacactgtgacctacactggctctgtcgtcagtcaggtctctgccggtgtgtacgcaactgttcgcttcgatcagtatgacatccataatctctggactattgagaagacctggtacgctcgtcatgcgacgcttcacaacggcaagaagatcagcatcaataacgtgacagaaatggcccctaccagcccgatcaagactaactgagcgatcgccagcagaacacgcgctgagggcccaaatcaccagtctctctctacaaatctatctctctctatttttctccagaataatgtgtgagtagttcccagataagggaattagggttcttatagggtttcgctcatgtgttgagcatataagaaacccttagtatgtatttgtatttgtaaaatacttctatcaataaaatttctaattcctaaaaccaaaatccagtcaaatcctaccacctcatttaaatagagtgaggttgatttgcggccgcacgtcctgcttggcctactaggccaacgcaggcgctggccgtgacggccacgagcgaactaggccttgggccgcatcgatcgtgaagtttctcatctaagcccccatttggacgtgaatgtagacacgtcgaaataaagatttccgaattagaataatttgtttattgctttcgcctataaatacgacggatcgtaatttgtcgttttatcaaaatgtactttcattttataataacgctgcggacatctacatttttgaattgaaaaaaaattggtaattactctttcttttttcaatataaacatgggaaatttgaaacttcctttttattattctaagaagtattaattccataatgaatgcatgaaggagttgttcaacaaattaatgaccaaaggtgaaattaaaagatttgtactcagaaattaatttttaatttaagtcgtgagacacgcttttgaaatgcattgaagttttttttttttaattaaatacaaatttccagataatgttagggacaaggcaaactagatggaaagacagtcattgaactaataagtaacagtaagaatatgtgtctttctttttattataacatacaaacacttagacattattaaaacagcccaagtttgtcgtttacaaagattgcaatctccatatcatgacaatacaatatactccatattgattgcattcataaaatatcattttacctcccttaccttaaatcccattcattcattagcatgagatttcaagtaaaattatgaactgaaaattagccaaatttattcaaaatttgaagaaaaaaaaccattttttctaataatttagtggcttaaattaaatctttcgaataattgaatgaccaaaatgtaattttattaataatttaatgacattggatgtaatatactcaatctaatatatcgagttaaaaaaaaaattctttggtacaaccagtgagttgtgtgaaatgcttcttaattaactatatgttcaattatatacattcaaaaacatacaaaatagccctgaaatatccaactttaatgggaccaatattatttttcatctatcgtaacatactacaacagttctatcaaaacatacaaaaattattgtttttttcttttttttttactcaggacccgcttagttcgactcatgaactagtttattttggatgtatatttttttatataatttcagtaaaatatatttcaaacattattgaagcaaagcaagaatgtaagtggtagagcagacagtatgttcactgatactgatgtcatatatatatatgttgggatgcaaggtttatagtgataaacaagaggttgaagatgttgtgtaagcatggtgccaagggaaaacatgaagaattggaccaccttctttacatgaatttggctgcatccttattctaacccattaatatttaaattataaaatattgtcattaagataacatgtcatttccttctctcattttctctgccaaatttgttctttttctccttctttttttttttcctttccatgtcttttaaagttctgattttgagagctgtctcctctatcttttatcttatttacataaaataaataaatttcatcataaatttaagtcccccaaaaaataaaaccataaaataaaataaaatctcagaaaaacctcccgttcgaaagcctctttcttttcttccacgggagcttaaagcttcgtcttgcaaaagtgggatagcacgaacttttgtgtgctttgtattgttattaattcttatatatttgccgtcaatccttatattttgaaaaaaaatttatgatttaatctctgtatttaaaaggttaaattttaagtttttcttttttttttaatttaaaaatctcagtctaaccattaacattattaatatttttctatcaaaatttatgaatttagcattttaattagattgtcctcatatgtcatgatatattaagttgacaaattttgattaaaattactagcaacgataatgattggattaggattgttaaattaaaaaataagaattgcatttttaaaaatattttttaaactgaaccggtgatcaaattggtcagatcatcggttcacaggcctaatcgtctaatcgattcgattaaaaattaataaaaattcaaaaaaaaattaaaatctcaattcaaccagttctcaatctaatcagttcaaagccactttccggactaattcccccaatcgattcttggtccggtccaattcaaataatactaattttttacttttaaagca

SEQ ID NO: 11 - DNA, 25 bp, Artificial
  Nucleotide sequence corresponding to a thermal amplification primer, SQ21940 used to identify cotton event MON 88702 DNA in a sample.
ctttcattttataataacgctgcgg

SEQ ID NO: 12 - DNA, 24 bp, Artificial
  Nucleotide sequence corresponding to a thermal amplification primer, SQ-50210 used to identify cotton event MON 88702 DNA in a sample.
aggaagtttcaaatttcccatgtt

SEQ ID NO: 13 - DNA, 22 bp, Artificial
  Nucleotide sequence corresponding to a probe, PB10344 used to identify cotton event MON 88702 DNA in a sample.
acatctacatttttgaattgaa

SEQ ID NO: 14 - DNA, 23 bp, Artificial
  Nucleotide sequence corresponding to a thermal amplification primer, SQ22496 used as an internal control in the event assay for MON 88702.
gaagaagcaccctctcatttacg

SEQ ID NO: 15 - DNA, 19 bp, Artificial
  Nucleotide sequence corresponding to a thermal amplification primer, SQ22497 used as an internal control in the event assay for MON 88702.
tggcagcacagcagatctg

SEQ ID NO: 16 - DNA, 20 bp, Artificial
  Nucleotide sequence corresponding to a probe, PB13032 used as an internal control in the event assay for MON 88702.
tgcgtccaatgcctgctcgc

SEQ ID NO: 17 - DNA, 24 bp, Artificial
  Nucleotide sequence corresponding to a thermal amplification primer, SQ50844 used in the zygosity assay for event MON 88702 DNA in a sample.
tcgcctataaatacgacggatcgt

SEQ ID NO: 18 - DNA, 20 bp, Artificial
  Nucleotide sequence corresponding to a probe, PB50279 used to identify cotton event MON 88702 allele in a sample for the zygosity assay.
aacgctgcggacatctacat

SEQ ID NO: 19 - DNA, 26 bp, Artificial
  Nucleotide sequence corresponding to a thermal amplifcation primer, SQ50843 used in the zygosity assay for event MON 88702 DNA in a sample which hybridizes to both the wild-type and MON 88702 alleles.
caactccttcatgcattcattatgga

SEQ ID NO: 20 - DNA, 25 bp, Artificial
  Nucleotide sequence corresponding to a thermal amplifcation primer, SQ50842 used int he zygosity assay for event MON 88702 DNA in a sample which hybridizes to only the wild-type DNA allele that does not contain the inserted MON 88702 transgene cassette.
ggtccctccacagtccacaaactat

SEQ ID NO: 21 - DNA, 21 bp, Artificial
  Nucleotide sequence corresponding to a probe, PB50278 used to identify the wild-type allel in the zygosity assay for event MON 88702 DNA in a sample.
ttctacatgtacttgctacca

SEQ ID NO: 22 - DNA, 101 bp, Artificial
  Nucleotide sequence representing the junction between the right T-DNA border sequence and the FMV 35S enhancer sequence within the transgene cassette used to transform DP393 cotton to produce cotton event MON 88702.
tcgcaattgaggtctgtcgaccctgcactaactataacggtcctaaggtagcgatacactggcgcgccaattctcagtccaaagcctcaacaaggtcaggg

SEQ ID NO: 23 - DNA, 77 bp, Artificial
  Nucleotide sequence representing the junction between the Arabidopsis thaliana HSP81.2 5' UTR and the TIC834_16 coding sequence within the transgene cassette used to transform DP393 cotton to produce cotton event MON 88702.
ttttttccgatctacgacacctgcaggcctcagcgctgtgcctgttgcgatcgcccatggctatcctagaccttaag

SEQ ID NO: 24 - DNA, 97 bp, Artificial
  Nucleotide sequence representing the junction between the TIC834_16 coding sequence and the 3' UTR within the transgene cassette used to transform DP393 cotton to produce cotton event MON 88702.
ccctaccagcccgatcaagactaactgagcgatcgccagcagaacacgcgctgagggcccaaatcaccagtctctctctacaaatctatctctctct

SEQ ID NO: 25 - DNA, 200 bp, Artificial
  Nucleotide sequence representing the junction between the 3' UTR and the left T-DNA border sequence within the transgene cassette used to transform DP393 cotton to produce cotton event MON 88702.
atttctaattcctaaaaccaaaatccagtcaaatcctaccacctcatttaaatagagtgaggttgatttgcggccgcacgtcctgcttggcctactaggccaacgcaggcgctggccgtgacggccacgagcgaactaggccttgggccgcatcgatcgtgaagtttctcatctaagcccccatttggacgtgaatgtag

SEQ ID NO: 26 - DNA, 921 bp, Artificial
  Nucleotide sequence representing the TIC834_16 coding sequence within the transgene cassette used to transform DP393 cotton to produce cotton event MON 88702.
atggctatcctagaccttaagtccctcgtgctgaacgccattaactactggggccctaagaacaacaacggcatccagggcggtgacttcggctaccccatctctgagaagcagatcgacactagcatcattacctccacccaccctcgcttgatcccccacgatcttactatcccgcagaaccttgagaccatcttcaccacaacgcaggtgctcaccaataacactgacctccagcaatcccagaccgtgagctttgcgaagaagaccactaccacgaccgcaactagcacgaccaacggttggacagaaggaggcaagatcagcgacacgctggaggagaaagtttcggttagcattccgttcatcggtgagggtggcgggaagaactcgactaccatagaggccaacttcgcacacaactctagcaccactacctcccaggaagcaagcactgacattgagtggaacattagccaaccggtccttgtgcctccccgcaaacaggttgttgccactctcgttatcatgggtggcaacttcactattcctatggatcttatgactaccattgactctactgagcactactctggctaccccattctcacttggatctcttctcctgacaatagctacagcggtcgattcatgtcatggtacttcgctaactggccgaatctcccttctggctttggtcctcttaactctgataacactgtgacctacactggctctgtcgtcagtcaggtctctgccggtgtgtacgcaactgttcgcttcgatcagtatgacatccataatctctggactattgagaagacctggtacgctcgtcatgcgacgcttcacaacggcaagaagatcagcatcaataacgtgacagaaatggcccctaccagcccgatcaagactaactga

SEQ ID NO: 27 - DNA, 3598 bp, Artificial
  Nucleotide sequence representing the transgene cassette comprised within the binary plasmid transformation vector used to transform DP393 cotton to produce cotton event MON 88702.
cgaagctcggtcccgtgggtgttctgtcgtctcgttgtacaacgaaatccattcccattccgcgctcaagatggcttcccctcggcagttcatcagggctaaatcaatctagccgacttgtccggtgaaatgggctgcactccaacagaaacaatcaaacaaacatacacagcgacttattcacacgagctcaaattacaacggtatatatcctgccagtcagcatcatcacaccaaaagttaggcccgaatagtttgaaattagaaagctcgcaattgaggtctgtcgaccctgcactaactataacggtcctaaggtagcgatacactggcgcgccaattctcagtccaaagcctcaacaaggtcagggtacagagtctccaaaccattagccaaaagctacaggagatcaatgaagaatcttcaatcaaagtaaactactgttccagcacatgcatcatggtcagtaagtttcagaaaaagacatccaccgaagacttaaagttagtgggcatctttgaaagtaatcttgtcaacatcgagcagctggcttgtggggaccagacaaaaaaggaatggtgcagaattgttaggcgcacctaccaaaagcatctttgcctttattgcaaagataaagcagattcctctagtacaagtggggaacaaaataacgtggaaaagagctgtcctgacagcccactcactaatgcgtatgacgaacgcagtgacgaccacaaaagaattagcttgcctgcaggattagcttagatcgggcttaattaaggcgcgccggccaagtcggccgcggccgcaagcttacttgcgacagaaacagctttgatatattattactcacccgttatcgatatggaatatatactttaagaactcactaaatcatatccttcatgtcggtttaaagattagtcacgtatctgcacattctgtaagtatagtaatctcataaaaaacctggtctctgttctctgtgaatccataggttattgcactggcgtactactgtatatcatatttccctggtggatcatcgggaatgaagttcctcagttctactcttacctcctctgtcttccgaatgtttgggagatgagctttcgctttgacctatgcaaagaaaataacttgattctctcgtgtataaagaaagatgaaagatcttcaacagtggttaaatgacaaatctggtaaaatatgttggtccaatggctcaaagacagttttgttataaatttcctatattgatactttctgctaaattggttcaaaacttcaaatcactagccactggatgaggtatggaacttgaagagttgcttggtggatacattctctaatctagggtaagtcgttagcttcaatgtcttactgtgaattattacatcagaattaagaaagttattacacgtatgttttcactgagtttactacactggcaatgtggcatacatctcttactgcaaattgcagacaagtggtcaatcaaatcttttttagttgggcccaaaatgtctgttattggatacgttgggccttaaaatggcccccatcagtcaaaaacatcactgcttggagaaggatctagaaaaacttgcaagttagttcaaacaaaataaaggaaaaagaacgatctagaagaaagaaaaaaaaaggaaaagaaacccttatggaggttcccacaccactctatatataataacatccttctcctaaatcccgcatcagtacttctctctgctctcaagataattttgttctctcaatttcattcttaaaccctagttcttcgattttttccgatctacgacacctgcaggcctcagcgctgtgcctgttgcgatcgcccatggctatcctagaccttaagtccctcgtgctgaacgccattaactactggggccctaagaacaacaacggcatccagggcggtgacttcggctaccccatctctgagaagcagatcgacactagcatcattacctccacccaccctcgcttgatcccccacgatcttactatcccgcagaaccttgagaccatcttcaccacaacgcaggtgctcaccaataacactgacctccagcaatcccagaccgtgagctttgcgaagaagaccactaccacgaccgcaactagcacgaccaacggttggacagaaggaggcaagatcagcgacacgctggaggagaaagtttcggttagcattccgttcatcggtgagggtggcgggaagaactcgactaccatagaggccaacttcgcacacaactctagcaccactacctcccaggaagcaagcactgacattgagtggaacattagccaaccggtccttgtgcctccccgcaaacaggttgttgccactctcgttatcatgggtggcaacttcactattcctatggatcttatgactaccattgactctactgagcactactctggctaccccattctcacttggatctcttctcctgacaatagctacagcggtcgattcatgtcatggtacttcgctaactggccgaatctcccttctggctttggtcctcttaactctgataacactgtgacctacactggctctgtcgtcagtcaggtctctgccggtgtgtacgcaactgttcgcttcgatcagtatgacatccataatctctggactattgagaagacctggtacgctcgtcatgcgacgcttcacaacggcaagaagatcagcatcaataacgtgacagaaatggcccctaccagcccgatcaagactaactgagcgatcgccagcagaacacgcgctgagggcccaaatcaccagtctctctctacaaatctatctctctctatttttctccagaataatgtgtgagtagttcccagataagggaattagggttcttatagggtttcgctcatgtgttgagcatataagaaacccttagtatgtatttgtatttgtaaaatacttctatcaataaaatttctaattcctaaaaccaaaatccagtcaaatcctaccacctcatttaaatagagtgaggttgatttgcggccgcacgtcctgcttggcctactaggccaacgcaggcgctggccgtgacggccacgagcgaactaggccttgggccgcatcgatcgtgaagtttctcatctaagcccccatttggacgtgaatgtagacacgtcgaaataaagatttccgaattagaataatttgtttattgctttcgcctataaatacgacggatcgtaatttgtcgttttatcaaaatgtactttcattttataataacgctgcggacatctacatttttgaattgaaaaaaaattggtaattactctttctttttctccatattgaccatcatactcattgctgatccatgtagatttcccggacatgaagccatttacaattgaatatatcctgccgccgctgccgctttgcacccggtggagcttgcatgttggtttctacgcagaactgagccggttaggcagataatttccattgagaactgagccatgtgcaccttccccccaacacggtgagcgacggggcaacggagtgatccacatgggactttt